European Patent Application EP 4 733 416 A1, published April 29, 2026. Title: Zestaw starterów do wykrywania mutacji onkogennych w DNA, sposób wykrywania mutacji onkogennych w DNA i jego zastosowanie do oceny nowotworowego pochodzenia komórek. Applicant: Gdański Uniwersytet Medyczny. The sequence listing filed with the application follows.

SEQUENCE LISTING (69 sequences)

SEQ ID NO: 1 - DNA, 30 bp, synthetic construct
  misc_feature 1..30: note = sekwencja nukleotydowa startera forward do wykrywania polimorfizmu w genie TP53
  source 1..30: mol_type = other DNA
acgttggatgagattctcttcctctgtgcg

SEQ ID NO: 2 - DNA, 30 bp, synthetic construct
  misc_feature 1..30: note = Sekwencja nukleotydowa startera forward do wykrywania polimorfizmu z genie TP53
  source 1..30: mol_type = other DNA
acgttggatgccaccatccactacaactac

SEQ ID NO: 3 - DNA, 30 bp, synthetic construct
  misc_feature 1..30: note = Sekwencja nukleotydowa startera forward do wykrywania polimorfizmu w genie TP53
  source 1..30: mol_type = other DNA
acgttggatgtccagtgtgatgatggtgag

SEQ ID NO: 4 - DNA, 30 bp, synthetic construct; identical to SEQ ID NO: 1
  misc_feature 1..30: note = Sekwencja nukleotydowa startera forward do wykrywania polimorfizum w genie TP53
  source 1..30: mol_type = other DNA

SEQ ID NO: 5 - DNA, 30 bp, synthetic construct
  misc_feature 1..30: note = rs397516436F
  source 1..30: mol_type = other DNA
acgttggatgagttgcaaaccagacctcag

SEQ ID NO: 6 - DNA, 29 bp, synthetic construct
  misc_feature 1..29: note = rs28934578F
  source 1..29: mol_type = other DNA
acgttggatgtgctcaccatcgctatctg

SEQ ID NO: 7 - DNA, 30 bp, synthetic construct; identical to SEQ ID NO: 5
  misc_feature 1..30: note = rs121912666F
  source 1..30: mol_type = other DNA

SEQ ID NO: 8 - DNA, 30 bp, synthetic construct
  misc_feature 1..30: note = Sekwencja nukleotydowa startera forward do wykrywania polimorfizmu w genie PIK3CA
  source 1..30: mol_type = other DNA
acgttggatgaactgagcaagaggctttgg

SEQ ID NO: 9 - DNA, 30 bp, synthetic construct
  misc_feature 1..30: note = Sekwencja nukleotydowa startera forward do wykrywania polimorfizum w genie PIK3CA
  source 1..30: mol_type = other DNA
acgttggatgtagcacttacctgtgactcc

SEQ ID NO: 10 - DNA, 30 bp, synthetic construct; identical to SEQ ID NO: 9
  misc_feature 1..30: note = Sekwencja nukleotydowa startera forward do wykrywania polimorfizmu w genie PIK3CA
  source 1..30: mol_type = other DNA

SEQ ID NO: 11 - DNA, 30 bp, synthetic construct
  misc_feature 1..30: note = rs121913284F
  source 1..30: mol_type = other DNA
acgttggatggggttataaatagtgcactc

SEQ ID NO: 12 - DNA, 30 bp, synthetic construct; identical to SEQ ID NO: 8
  misc_feature 1..30: note = rs121913277F
  source 1..30: mol_type = other DNA

SEQ ID NO: 13 - DNA, 30 bp, synthetic construct; identical to SEQ ID NO: 9
  misc_feature 1..30: note = rs121913274F
  source 1..30: mol_type = other DNA

SEQ ID NO: 14 - DNA, 30 bp, synthetic construct
  misc_feature 1..30: note = rs121913286F
  source 1..30: mol_type = other DNA
acgttggatgtacacgagatcctctctctg

SEQ ID NO: 15 - DNA, 30 bp, synthetic construct
  misc_feature 1..30: note = rs1057519816F
  source 1..30: mol_type = other DNA
acgttggatgtcctgatctccttagacaac

SEQ ID NO: 16 - DNA, 29 bp, synthetic construct
  misc_feature 1..29: note = rs121913471F
  source 1..29: mol_type = other DNA
acgttggatgcgtggatgtcaggcagatg

SEQ ID NO: 17 - DNA, 30 bp, synthetic construct
  misc_feature 1..30: note = rs121913470F
  source 1..30: mol_type = other DNA
acgttggatggggcttacgtctaagatttc

SEQ ID NO: 18 - DNA, 30 bp, synthetic construct
  misc_feature 1..30: note = rs796065354F
  source 1..30: mol_type = other DNA
acgttggatgaagcccgctcatgatcaaac

SEQ ID NO: 19 - DNA, 30 bp, synthetic construct
  misc_feature 1..30: note = rs1057519717F
  source 1..30: mol_type = other DNA
acgttggatgcagcatgaagtgcaagaacg

SEQ ID NO: 20 - DNA, 30 bp, synthetic construct; identical to SEQ ID NO: 19
  misc_feature 1..30: note = rs2152506534F
  source 1..30: mol_type = other DNA

SEQ ID NO: 21 - DNA, 30 bp, synthetic construct; identical to SEQ ID NO: 19
  misc_feature 1..30: note = rs2152506541F
  source 1..30: mol_type = other DNA

SEQ ID NO: 22 - DNA, 29 bp, synthetic construct
  misc_feature 1..29: note = rs1962456814F
  source 1..29: mol_type = other DNA
acgttggatgccggttccatctacctttc

SEQ ID NO: 23 - DNA, 29 bp, synthetic construct
  misc_feature 1..29: note = rs121434592F
  source 1..29: mol_type = other DNA
acgttggatgtctgacgggtagagtgtgc

SEQ ID NO: 24 - DNA, 30 bp, synthetic construct
  misc_feature 1..30: note = Sekwencja nukleotydowa startera reverse do wykrywania polimorfizmu w genie TP53
  source 1..30: mol_type = other DNA
acgttggatgagtggtaatctactgggacg

SEQ ID NO: 25 - DNA, 30 bp, synthetic construct; identical to SEQ ID NO: 3
  misc_feature 1..30: note = Sekwencja nukleotydowa startera reverse do wykrywania polimorfizmu w genie TP53
  source 1..30: mol_type = other DNA

SEQ ID NO: 26 - DNA, 30 bp, synthetic construct; identical to SEQ ID NO: 2
  misc_feature 1..30: note = Sekwencja nukleotydowa startera reverse do wykrywania polimorfizmu w genie TP53
  source 1..30: mol_type = other DNA

SEQ ID NO: 27 - DNA, 30 bp, synthetic construct; identical to SEQ ID NO: 24
  misc_feature 1..30: note = Sekwencja nukleotydowa startera reverse do wykrywania polimorfizmu w genie TP53
  source 1..30: mol_type = other DNA

SEQ ID NO: 28 - DNA, 30 bp, synthetic construct
  misc_feature 1..30: note = rs397516436R
  source 1..30: mol_type = other DNA
acgttggatggtgtggagtatttggatgac

SEQ ID NO: 29 - DNA, 30 bp, synthetic construct
  misc_feature 1..30: note = rs28934578R
  source 1..30: mol_type = other DNA
acgttggatgccatctacaagcagtcacag

SEQ ID NO: 30 - DNA, 30 bp, synthetic construct; identical to SEQ ID NO: 28
  misc_feature 1..30: note = rs121912666R
  source 1..30: mol_type = other DNA

SEQ ID NO: 31 - DNA, 30 bp, synthetic construct
  misc_feature 1..30: note = Sekwencja nukleotydowa startera reverse do wykrywania polimorfizmu w genie PIK3CA
  source 1..30: mol_type = other DNA
acgttggatgtccatttttgttgtccagcc

SEQ ID NO: 32 - DNA, 30 bp, synthetic construct
  misc_feature 1..30: note = Sekwencja nukleotydowa startera reverse do wykrywania polimorfizmu w genie PIK3CA
  source 1..30: mol_type = other DNA
acgttggatggcaatttctacacgagatcc

SEQ ID NO: 33 - DNA, 30 bp, synthetic construct; identical to SEQ ID NO: 14
  misc_feature 1..30: note = Sekwencja nukleotydowa startera reverse do amplifikacji polimorfizmu w genie PIK3CA
  source 1..30: mol_type = other DNA

SEQ ID NO: 34 - DNA, 30 bp, synthetic construct
  misc_feature 1..30: note = rs121913284R
  source 1..30: mol_type = other DNA
acgttggatgcatcagcatttgactttacc

SEQ ID NO: 35 - DNA, 29 bp, synthetic construct
  misc_feature 1..29: note = rs121913277R
  source 1..29: mol_type = other DNA
acgttggatgttgtgtggaagatccaatc

SEQ ID NO: 36 - DNA, 30 bp, synthetic construct; identical to SEQ ID NO: 14
  misc_feature 1..30: note = rs121913274R
  source 1..30: mol_type = other DNA

SEQ ID NO: 37 - DNA, 30 bp, synthetic construct; identical to SEQ ID NO: 9
  misc_feature 1..30: note = rs121913286R
  source 1..30: mol_type = other DNA

SEQ ID NO: 38 - DNA, 29 bp, synthetic construct
  misc_feature 1..29: note = rs1057519816R
  source 1..29: mol_type = other DNA
acgttggatgtcacctcttggttgtgcag

SEQ ID NO: 39 - DNA, 29 bp, synthetic construct
  misc_feature 1..29: note = rs121913471R
  source 1..29: mol_type = other DNA
acgttggatgccaggaagcatacgtgatg

SEQ ID NO: 40 - DNA, 29 bp, synthetic construct
  misc_feature 1..29: note = rs121913470R
  source 1..29: mol_type = other DNA
acgttggatggaaaattccagtggccatc

SEQ ID NO: 41 - DNA, 30 bp, synthetic construct
  misc_feature 1..30: note = rs796065354R
  source 1..30: mol_type = other DNA
acgttggatgaacaaggcactgaccatctg

SEQ ID NO: 42 - DNA, 29 bp, synthetic construct
  misc_feature 1..29: note = rs1057519717R
  source 1..29: mol_type = other DNA
acgttggatggctagtgggcgcatgtagg

SEQ ID NO: 43 - DNA, 29 bp, synthetic construct
  misc_feature 1..29: note = rs2152506534R
  source 1..29: mol_type = other DNA
acgttggatggctagtgggcgcatgtagg

SEQ ID NO: 44 - DNA, 29 bp, synthetic construct
  misc_feature 1..29: note = rs2152506541R
  source 1..29: mol_type = other DNA
acgttggatggctagtgggcgcatgtagg

SEQ ID NO: 45 - DNA, 30 bp, synthetic construct
  misc_feature 1..30: note = rs1962456814R
  source 1..30: mol_type = other DNA
acgttggatgtgtagctctcggcgtcaaag

SEQ ID NO: 46 - DNA, 30 bp, synthetic construct
  misc_feature 1..30: note = rs121434592R
  source 1..30: mol_type = other DNA
acgttggatgttcttgaggaggaagtagcg

SEQ ID NO: 47 - DNA, 17 bp, synthetic construct
  misc_feature 1..17: note = Sekwencja startera r nicuj cego do wykrywania polimorfizmu w genie TP53
  source 1..17: mol_type = other DNA
ggacagctttgaggtgc

SEQ ID NO: 48 - DNA, 16 bp, synthetic construct
  misc_feature 1..16: note = Sekwencja startera r nicuj cego do wykrywania polimorfizmu w genie TP53
  source 1..16: mol_type = other DNA
ttgaggatgggcctcc

SEQ ID NO: 49 - DNA, 15 bp, synthetic construct
  misc_feature 1..15: note = Sekwencja nukleotydowa startera r nicuj cego do wykrywania polimorfizmu w genie TP53
  source 1..15: mol_type = other DNA
tgggcggcatgaacc

SEQ ID NO: 50 - DNA, 18 bp, synthetic construct
  misc_feature 1..18: note = Sekwencja nukleotydowa startera r nicuj cego do wykrywania polimorfizmu w genie TP53
  source 1..18: mol_type = other DNA
cggaacagctttgaggtg

SEQ ID NO: 51 - DNA, 17 bp, synthetic construct
  misc_feature 1..17: note = rs397516436D
  source 1..17: mol_type = other DNA
atgacagaaacactttt

SEQ ID NO: 52 - DNA, 15 bp, synthetic construct
  misc_feature 1..15: note = rs28934578D
  source 1..15: mol_type = other DNA
cggaggttgtgaggc

SEQ ID NO: 53 - DNA, 18 bp, synthetic construct
  misc_feature 1..18: note = rs121912666D
  source 1..18: mol_type = other DNA
atagtgtggtggtgccct

SEQ ID NO: 54 - DNA, 15 bp, synthetic construct
  misc_feature 1..15: note = Sekwencja nukleotydowa startera r nicuj cego do wykrywania polimorfizmu w genie PIK3CA
  source 1..15: mol_type = other DNA
gtccagccaccatga

SEQ ID NO: 55 - DNA, 17 bp, synthetic construct
  misc_feature 1..17: note = Sekwencja nukleotydowa startera r nicuj cego do wykrywania polimorfizmu w genie PIK3CA
  source 1..17: mol_type = other DNA
cacgagatcctctctct

SEQ ID NO: 56 - DNA, 18 bp, synthetic construct
  misc_feature 1..18: note = Sekwencja nukleotydowa startera r nicuj cego do wykrywania polimorfizmu w genie PIK3CA
  source 1..18: mol_type = other DNA
cctctctctgaaatcact

SEQ ID NO: 57 - DNA, 25 bp, synthetic construct
  misc_feature 1..25: note = rs121913284D
  source 1..25: mol_type = other DNA
ccttatcaatgtctcgaatatttac

SEQ ID NO: 58 - DNA, 19 bp, synthetic construct
  misc_feature 1..19: note = rs121913277D
  source 1..19: mol_type = other DNA
atttttgttgtccagccac

SEQ ID NO: 59 - DNA, 17 bp, synthetic construct
  misc_feature 1..17: note = rs121913274D
  source 1..17: mol_type = other DNA
tctctctgaaatcactg

SEQ ID NO: 60 - DNA, 16 bp, synthetic construct
  misc_feature 1..16: note = rs121913286D
  source 1..16: mol_type = other DNA
agaaaatctttctcct

SEQ ID NO: 61 - DNA, 18 bp, synthetic construct
  misc_feature 1..18: note = rs1057519816D
  source 1..18: mol_type = other DNA
gggcagacgagggtgcag

SEQ ID NO: 62 - DNA, 20 bp, synthetic construct
  misc_feature 1..20: note = rs121913471D
  source 1..20: mol_type = other DNA
aagcatacgtgatggctggt

SEQ ID NO: 63 - DNA, 16 bp, synthetic construct
  misc_feature 1..16: note = rs121913470D
  source 1..16: mol_type = other DNA
gtggccatcaaagtgt

SEQ ID NO: 64 - DNA, 19 bp, synthetic construct
  misc_feature 1..19: note = rs796065354D
  source 1..19: mol_type = other DNA
ggacaaggccaggctgttc

SEQ ID NO: 65 - DNA, 22 bp, synthetic construct
  misc_feature 1..22: note = rs1057519717D
  source 1..22: mol_type = other DNA
catctccagcagcaggtcatag

SEQ ID NO: 66 - DNA, 15 bp, synthetic construct
  misc_feature 1..15: note = rs2152506534D
  source 1..15: mol_type = other DNA
ccagcagcaggtcat

SEQ ID NO: 67 - DNA, 18 bp, synthetic construct
  misc_feature 1..18: note = rs2152506541D
  source 1..18: mol_type = other DNA
atctccagcagcaggtca

SEQ ID NO: 68 - DNA, 22 bp, synthetic construct
  misc_feature 1..22: note = rs1962456814D
  source 1..22: mol_type = other DNA
gggtggcagggctccggctcct

SEQ ID NO: 69 - DNA, 24 bp, synthetic construct
  misc_feature 1..24: note = rs121434592D
  source 1..24: mol_type = other DNA
gtggccgccaggtcttgatgtact